European Patent Application EP 4 130 041 A1, published February 8, 2023. Title: Anti-PD-L1 and PD-L2 antibody and derivatives and use thereof. Applicant: BIOTHEUS INC. Application PCT/CN2021/084196. The sequence listing filed with the application follows.

SEQUENCE LISTING (71 sequences)

SEQ ID NO: 1 - protein, 119 aa, artificial sequence
  D-Na-58 VHH chain amino acid sequence
QVQLVESGGGLVQAGGSLTLSCTASGRTFSSYAMAWFRQAPGKERELLVTISRSGSTTYYLDSVKGRFTISRDNAKNTVYLQMNSLKPEDTAVYYCAAKRSLQDEVYYWGQGTQVTVSS

SEQ ID NO: 2 - protein, 119 aa, artificial sequence
  D-Na-64 VHH chain amino acid sequence
EVQLVESGGGLVQPGGSLRLSCAASGRTFSSMTIGWFRQTPGKEREFVAGIGWSTSKTVYKDSVKGRFTISTDNAKKTVYLQMNNLKPEDTAVYYCAADSMNRGQFDYWGQGTQVTVSS

SEQ ID NO: 3 - protein, 119 aa, artificial sequence
  D-Na-96 VHH chain amino acid sequence
QVQLVESGGGLVQAGASLRLSCAASGRTFSSMTIGWFRQTPGKEREFVAGIGWTSGLTVYADSVKGRFTISRDNAEKTMYLHMNNLKPEDTSVYYCAADSMNRGQFDYWGQGTQVTVSS

SEQ ID NO: 4 - protein, 124 aa, artificial sequence
  D-Na-67 VHH chain amino acid sequence
QVQLVESGGGLVQAGGSLRLSCAASGGLTFINYAMGWFRQAPGKEREFVAAISRFGGTTSYADSVKDRFSITRDVAKDTVYLQTNSLKPEDTAVYYCAANSRILSRTAADYDYWGQGTQVTVSS

SEQ ID NO: 5 - protein, 125 aa, artificial sequence
  D-Na-78 VHH chain amino acid sequence
QVQLVESGGGLVQAGGSLRLSCEASGVISINYAMAWFRQAPGKEREFVAAISRFGVTTSYADSVKDRFSIGITRDNAKDTMYLQTKSLKPEDTAVYYCAANSRILSRTAKDYDYWGQGTQVTVSS

SEQ ID NO: 6 - protein, 122 aa, artificial sequence
  D-Na-80 VHH chain amino acid sequence
EVQLVESGGGLVQAGGSLRLSCAVSGVSFINYAMGWFRQAPGKEREFVAAISRFGGTTSYADSVKDRFSITTDTKDTVYLQTNSLKPEDTAVYYCAANSRILSRTAKDYDYWGQGTQVTVSS

SEQ ID NO: 7 - protein, 123 aa, artificial sequence
  D-Na-87 VHH chain amino acid sequence
QVQLVESGGGLVQPGGSLRLSCAASGFAFDAYAMTWVRQAPGKGLEFLSRIYSHGSKIIYAGSVKGRFTIFRDNAKNTVYLQMNSLKPEDTAVYYCAAGPDNIPTTGEKYDFWGQGTQVTVSS

SEQ ID NO: 8 - protein, 123 aa, artificial sequence
  D-Na-89 VHH chain amino acid sequence
QVQLVESGGGLVQAGGSLRLSCAASGLTFINYAMGWFRQAPGKEREFVAAISWAGGTTSYADSVKDRFSITRDSAKDTVYLQTNSLKPEDTAVYYCAANSRILSRTAKDYDYWGQGTEVTVSS

SEQ ID NO: 9 - protein, 123 aa, artificial sequence
  D-Na-90 VHH chain amino acid sequence
QVQLVESGGGLVQAGGSLRLSCAASGLTFINYAMGWFRQAPGKEREFVAAISWAGGTTSYADSVKDRFSITRDSAKDTVYLQTNSLKPEDTAVYYCAANSRILSRTAKDYDYWGQGTQVTVSS

SEQ ID NO: 10 - protein, 119 aa, artificial sequence
  D-Ye-10 VHH chain amino acid sequence
QVQLQESGGGLVQAGASLRLSCASSGRTFSSMTIGWFRQTPGKEREFVAGIGWSTSKTVYKDSVKGRFTISTDNAKKTVYLQMNNLKPEDTAVYYCAEDSMNRGQFDYWGQGTQVTVSS

SEQ ID NO: 11 - protein, 116 aa, artificial sequence
  D-Ye-22 VHH chain amino acid sequence
QVQLQESGGGLVQAGDSLRLSCIGSRRTFTMAWFRQAPGKEREFVAGIWGPADHTIYANSVKGRFACSRDDSTNTIFLQMNSLELEDTALYLCAAADSSGDDFEYWGQGTQVTVSS

SEQ ID NO: 12 - protein, 123 aa, artificial sequence
  D-Ye-29 VHH chain amino acid sequence
QVQLQESGGGLVQPGGSLRLSCAASGSEFSFIPTGWYRQTPGKQRDLVAVFTSGGLTNYADSVKGRFTISRNNTKNIVYLQMNSLKPEDTAVYYCSGVPGPHYNGPTSGINYWGQGTQVTVSS

SEQ ID NO: 13 - protein, 119 aa, artificial sequence
  D-Ye-31 VHH chain amino acid sequence
QVQLQESGGGLVQAGGSLGLSCAASGRTFSSMTIGWFRQTPGKEREFVAGIGWSTSKTVYKDSVKGRFTISTDNAKKTVYLQMNNLKPEDTAVYYCAADSMNRGQFDYWGQGTQVTVSS

SEQ ID NO: 14 - protein, 112 aa, artificial sequence
  D-Ye-32 VHH chain amino acid sequence
QVQLQESGGGLVQAGGSLRLSCAASGSVGSINAMAWFRQAPGKQRDVVAHMPSGGSTHYADSVKGRFTVSRDNAKNTVYLQMNSLKAEDTAVYYCWAAGLGWGQGTQVTVSS

SEQ ID NO: 15 - protein, 123 aa, artificial sequence
  HZ-D-Ye-29-3 VHH chain amino acid sequence
EVQLLESGGGLVQPGGSLRLSCAASGSEFSFIPTGWYRQAPGKQRELVAVFTSGGLTNYADSVKGRFTISRDNSKNTVYLQMNSLRAEDTAVYYCSGVPGPHYNGPTSGINYWGQGTQVTVSS

SEQ ID NO: 16 - protein, 119 aa, artificial sequence
  HZ-D-Na-96-1 VHH chain amino acid sequence
EVQLVESGGGLVQPGGSLRLSCAASGRTFSSMTIGWFRQAPGKGLEFVSGIGWTSGLTVYADSVKGRFTISRDNAKNSMYLQMNSLRAEDTAVYYCAADSMNRGQFDYWGQGTLVTVSS

SEQ ID NO: 17 - protein, 119 aa, artificial sequence
  HZ-D-Na-96-2 VHH chain amino acid sequence
EVQLVESGGGLVQPGGSLRLSCAASGRTFSSMTIGWFRQAPGKGLEFVSGIGWTSGLTVYADSVKGRFTISRDNAKNSLYLQMNSLKPEDTAVYYCAADSMNRGQFDYWGQGTLVTVSS

SEQ ID NO: 18 - protein, 119 aa, artificial sequence
  HZ-D-Na-96-3 VHH chain amino acid sequence
EVQLVESGGGLVQPGGSLRLSCAASGRTFSSMTIGWFRQAPGKEREFVSGIGWTSGLTVYADSVKGRFTISRDNAKNSMYLQMNSLKPEDTAVYYCAADSMNRGQFDYWGQGTLVTVSS

SEQ ID NO: 19 - protein, 124 aa, artificial sequence
  K-Yr-13&14-02 VHH chain amino acid sequence
QVQLVESGGGLVKAGDSLRLSCAASGHTFIIYAIGWFRQAPGKEREFVATINWSGSMTNYTDSVKGRFTISRDNAKNTVYLQMNSLKPDDTAIYYCAAYVGATISTAHSRYDYWGQGTQVTVSS

SEQ ID NO: 20 - protein, 124 aa, artificial sequence
  K-Yr-13&14-09 VHH chain amino acid sequence
QVQLVESGGGLVKAGDSLRLSCAASGRTFTIYAIGWFRQAPGKEREFVATINWSGSMTNYTDSVKGRFTISRDNAKNTVYLQMNSLKPDDTAIYYCAAYVGATISTAHSRYDYWGQGTLVTVSA

SEQ ID NO: 21 - protein, 124 aa, artificial sequence
  K-Yr-13&14-16 VHH chain amino acid sequence
EVQLVESGGGLVQAGGSLRLSCAASTRTFITYAMGWFRQAPGKEREFVASINWSGASTYYADSVKGRFTISRHNAKNTVYLQMNSLKPEDTAVYYCAAALSAVVVTQILDYDYWGQGTLVTVSS

SEQ ID NO: 22 - protein, 124 aa, artificial sequence
  HZ-K-Yr-13&14-02-3 VHH chain amino acid sequence
QVQLVESGGGLVKPGGSLRLSCAASGHTFIIYAIGWFRQAPGKGLEFVATINWSGSMTNYADSVKGRFTISRDNAKNTVYLQMNSLKPDDTAVYYCAAYVGATISTAHSRYDYWGQGTLVTVSS

SEQ ID NO: 23 - protein, 490 aa, artificial sequence
  Bi-201 amino acid sequence
QVQLVESGGGLVKPGGSLRLSCAASGHTFIIYAIGWFRQAPGKGLEFVATINWSGSMTNYADSVKGRFTISRDNAKNTVYLQMNSLKPDDTAVYYCAAYVGATISTAHSRYDYWGQGTLVTVSSDKTHTCPPCPAPEAAGGPSVFLFPPKPKDTLMISRTPEVTCVVVDVSHEDPEVKFNWYVDGVEVHNAKTKPREEQYNSTYRVVSVLTVLHQDWLNGKEYKCKVSNKALPAPIEKTISKAKGQPREPQVYTLPPSREEMTKNQVSLTCLVKGFYPSDIAVEWESNGQPENNYKTTPPVLDSDGSFFLYSKLTVDKSRWQQGNVFSCSVMHEALHNHYTQKSLSLSPGGGGGSGGGGSGGGGSGGGGSGEVQLVESGGGLVQPGGSLRLSCAASGRTFSSMTIGWFRQAPGKGLEFVSGIGWTSGLTVYADSVKGRFTISRDNAKNSMYLQMNSLRAEDTAVYYCAADSMNRGQFDYWGQGTLVTVSS

SEQ ID NO: 24 - protein, 490 aa, artificial sequence
  Bi-202 amino acid sequence
QVQLVESGGGLVKPGGSLRLSCAASGHTFIIYAIGWFRQAPGKGLEFVATINWSGSMTNYADSVKGRFTISRDNAKNTVYLQMNSLKPDDTAVYYCAAYVGATISTAHSRYDYWGQGTLVTVSSGGGGGSGGGGSGGGGSGGGGSGEVQLVESGGGLVQPGGSLRLSCAASGRTFSSMTIGWFRQAPGKGLEFVSGIGWTSGLTVYADSVKGRFTISRDNAKNSMYLQMNSLRAEDTAVYYCAADSMNRGQFDYWGQGTLVTVSSDKTHTCPPCPAPEAAGGPSVFLFPPKPKDTLMISRTPEVTCVVVDVSHEDPEVKFNWYVDGVEVHNAKTKPREEQYNSTYRVVSVLTVLHQDWLNGKEYKCKVSNKALPAPIEKTISKAKGQPREPQVYTLPPSREEMTKNQVSLTCLVKGFYPSDIAVEWESNGQPENNYKTTPPVLDSDGSFFLYSKLTVDKSRWQQGNVFSCSVMHEALHNHYTQKSLSLSP

SEQ ID NO: 25 - protein, 452 aa, artificial sequence
  Bi-203 amino acid sequence
QVQLVESGGGLVKPGGSLRLSCAASGHTFIIYAIGWFRQAPGKGLEFVATINWSGSMTNYADSVKGRFTISRDNAKNTVYLQMNSLKPDDTAVYYCAAYVGATISTAHSRYDYWGQGTLVTVSSASTKGPSVFPLAPSSKSTSGGTAALGCLVKDYFPEPVTVSWNSGALTSGVHTFPAVLQSSGLYSLSSVVTVPSSSLGTQTYICNVNHKPSNTKVDKKVEPKSCDKTHTCPPCPAPEAAGGPSVFLFPPKPKDTLMISRTPEVTCVVVDVSHEDPEVKFNWYVDGVEVHNAKTKPREEQYNSTYRVVSVLTVLHQDWLNGKEYKCKVSNKALPAPIEKTISKAKGQPREPQVYTLPPSREEMTKNQVSLTCLVKGFYPSDIAVEWESNGQPENNYKTTPPVLDSDGSFFLYSKLTVDKSRWQQGNVFSCSVMHEALHNHYTQKSLSLSP

SEQ ID NO: 26 - protein, 226 aa, artificial sequence
  Bi-204 amino acid sequence
EVQLVESGGGLVQPGGSLRLSCAASGRTFSSMTIGWFRQAPGKGLEFVSGIGWTSGLTVYADSVKGRFTISRDNAKNSMYLQMNSLRAEDTAVYYCAADSMNRGQFDYWGQGTLVTVSSRTVAAPSVFIFPPSDEQLKSGTASVVCLLNNFYPREAKVQWKVDNALQSGNSQESVTEQDSKDSTYSLSSTLTLSKADYEKHKVYACEVTHQGLSSPVTKSFNRGEC

SEQ ID NO: 27 - protein, 21 aa, artificial sequence
  linker
GGGGSGGGGSGGGGSGGGGSG

SEQ ID NO: 28 - protein, 225 aa, artificial sequence
  Fc
DKTHTCPPCPAPEAAGGPSVFLFPPKPKDTLMISRTPEVTCVVVDVSHEDPEVKFNWYVDGVEVHNAKTKPREEQYNSTYRVVSVLTVLHQDWLNGKEYKCKVSNKALPAPIEKTISKAKGQPREPQVYTLPPSREEMTKNQVSLTCLVKGFYPSDIAVEWESNGQPENNYKTTPPVLDSDGSFFLYSKLTVDKSRWQQGNVFSCSVMHEALHNHYTQKSLSLSP

SEQ ID NO: 29 - protein, 103 aa, artificial sequence
  CH1
ASTKGPSVFPLAPSSKSTSGGTAALGCLVKDYFPEPVTVSWNSGALTSGVHTFPAVLQSSGLYSLSSVVTVPSSSLGTQTYICNVNHKPSNTKVDKKVEPKSC

SEQ ID NO: 30 - protein, 107 aa, artificial sequence [sequence omitted]

SEQ ID NO: 31 - DNA, 357 bp, artificial sequence
  D-Na-58 VHH chain nucleotide sequence
caggtgcagctcgtggagtcaggcggaggattggtgcaggctgggggctctctgacactctcctgtacagcctctggacgcaccttcagtagctatgccatggcctggttccgccaggctccagggaaggagcgtgagttattagtaactatcagcaggagtggtagtaccacttactatcttgactccgtgaagggccgattcaccatctccagagacaacgccaagaacacggtgtatctgcaaatgaacagcctgaaacctgaggacacggccgtttattactgtgcagcaaaaaggtctctccaagacgaagtttactactggggccaggggacccaggtcaccgtctcctca

SEQ ID NO: 32 - DNA, 357 bp, artificial sequence
  D-Na-64 VHH chain nucleotide sequence
gaggtgcagctcgtggagtcagggggaggcttggtgcagcctggggggtctctgagactctcctgcgcagcctctggacgcaccttcagtagcatgaccatcggctggttccgccaaactccagggaaggagcgtgagtttgtagcaggtattgggtggagtacgagtaaaacagtctacaaagactccgtgaagggccgattcaccatttccacagacaatgccaagaaaacggtgtatctgcaaatgaacaacctgaaacctgaggacacggccgtttattactgtgcagcagattcaatgaatagaggacagtttgactactggggccaggggacccaggtcaccgtctcctca

SEQ ID NO: 33 - DNA, 357 bp, artificial sequence
  D-Na-96 VHH chain nucleotide sequence
caggtgcagctcgtggagtccgggggaggattggtgcaggctggggcctctctgagactctcctgcgcagcctctggacgcaccttcagtagcatgaccatcggctggttccgccaaactccagggaaggagcgtgagtttgtagcaggtattgggtggacgagtggtctcacagtctatgcagactccgtgaagggccgattcaccatttccagagacaatgccgagaaaacgatgtatctgcacatgaacaatctgaaacctgaggacacgtccgtttattactgtgcagcagattcaatgaacagaggacagtttgactactggggccaggggacccaggtcaccgtctcctca

SEQ ID NO: 34 - DNA, 372 bp, artificial sequence
  D-Na-67 VHH chain nucleotide sequence
caggtgcagctcgtggagtctggtggaggattggtgcaggctgggggctctctgagactctcctgtgcagcctctggtggactcaccttcattaactatgccatgggctggttccgccaggctccagggaaggagcgtgagtttgtagcagctattagtcggtttggtggcactacatcctacgcagactccgtgaaggaccgattcagcatcactagagatgttgccaaagacacggtgtatttgcaaacgaacagcctgaaacctgaggacacggccgtttattactgtgcagcaaactcccgtattctgagtcgaaccgctgcggattacgattactggggccaggggacccaggtcaccgtctcctca

SEQ ID NO: 35 - DNA, 375 bp, artificial sequence
  D-Na-78 VHH chain nucleotide sequence
caggtgcagctcgtggagtccggcggaggattggtgcaggctgggggctctctgagactctcctgtgaagcctctggagtcatctccattaactatgccatggcctggttccgccaggctccagggaaggagcgtgagtttgtagctgctattagtcggtttggtgtaactacgagttacgcagactccgtgaaggaccgattcagcatcggcatcactagagataatgccaaagacacaatgtatctgcaaacgaagagcctgaaacctgaggacacggccgtttattattgtgcagcaaactcccgtattctgagtcgaaccgctaaggattatgattactggggccaggggacccaggtcaccgtctcctca

SEQ ID NO: 36 - DNA, 366 bp, artificial sequence
  D-Na-80 VHH chain nucleotide sequence
gaggtgcagctcgtggagtctggtggaggattggtgcaggctgggggctctctgagactctcctgtgcagtctctggagtctccttcattaactatgccatgggctggttccgccaggctccagggaaggagcgtgagtttgtagcagctattagtcggtttggtggcactacatcctacgcagactccgtgaaggaccgattcagcatcactacagataccaaagacacggtgtatctgcaaacgaacagcctgaaacctgaggacacggccgtttattattgtgcagcaaactcccgtattctgagtcgaaccgctaaggattatgattactggggccaggggacccaggtcaccgtctcctca

SEQ ID NO: 37 - DNA, 369 bp, artificial sequence
  D-Na-87 VHH chain nucleotide sequence
caggtgcagctcgtggagtctgggggaggcttggtgcagcctgggggttctctgagactctcctgtgcagcctctggattcgcttttgatgcctatgccatgacctgggtccgacaggctccagggaagggactggagtttttgtcccgtatttatagtcatggaagtaagatcatctacgcaggttccgtgaagggccgattcaccattttcagagacaacgccaagaacacggtgtatctgcaaatgaacagcctgaaacctgaggacacggccgtgtattactgtgcagctggtccggacaacataccgactacaggtgaaaagtatgacttctggggtcaggggacccaggtcaccgtctcctca

SEQ ID NO: 38 - DNA, 369 bp, artificial sequence
  D-Na-89 VHH chain nucleotide sequence
caggtgcagctcgtggagtcagggggaggattggtgcaggctgggggctctctgagactctcctgtgcagcctctggactcaccttcattaactatgccatgggctggttccgccaggctccagggaaggagcgtgagtttgtagcagctattagttgggctggtggcactacatcctacgcagactccgtgaaggaccgattcagcatcactagagactctgccaaagacacggtgtatctgcaaacgaacagcctgaaacctgaggacacggccgtttattattgtgcagcaaactcccgtattctgagtcgaaccgctaaggattatgattactggggccaggggaccgaggtcaccgtctcctca

SEQ ID NO: 39 - DNA, 369 bp, artificial sequence
  D-Na-90 VHH chain nucleotide sequence
caggtgcagctcgtggagtctgggggaggattggtgcaggctgggggctctctgagactctcctgtgcagcctctggactcaccttcattaactatgccatgggctggttccgccaggctccagggaaggagcgtgagtttgtagcagctattagttgggctggtggcactacatcctacgcagactccgtgaaggaccgattcagcatcactagagactctgccaaagacacggtgtatctgcaaacgaacagcctgaaacctgaggacacggccgtttattattgtgcagcaaactcccgtattctgagtcgaaccgctaaggattatgattactggggccaggggacccaggtcaccgtctcctca

SEQ ID NO: 40 - DNA, 357 bp, artificial sequence
  D-Ye-10 VHH chain nucleotide sequence
caggtgcagctgcaggagtctgggggaggattggtgcaggctggggcctctctgagactctcctgcgcatcctctggacgcaccttcagtagcatgaccatcggctggttccgccaaactccagggaaggagcgtgagtttgtagcaggtattgggtggagtacgagtaaaacagtctacaaagactccgtgaagggccgattcaccatttccacagacaatgccaagaaaacggtgtatctgcaaatgaacaacctgaaacctgaggacacggccgtttattactgtgcagaagattcaatgaatagaggacagtttgactactggggccaggggacccaggtcaccgtctccagt

SEQ ID NO: 41 - DNA, 348 bp, artificial sequence
  D-Ye-22 VHH chain nucleotide sequence
caggtgcagctgcaggagtctggaggaggattggtgcaggctggggactctctgagactctcctgtataggttctagacgtaccttcaccatggcctggttccgccaggctccagggaaggagcgtgaatttgtggcaggtatttggggtcctgcggatcacacaatctatgcaaactccgtgaagggccgattcgcctgctccagagacgattccacgaatacgatttttttgcaaatgaacagcctggaacttgaggacacggccctttatctctgtgcagcagcggactccagtggggatgactttgagtattggggccaggggacccaggtcaccgtctccagt

SEQ ID NO: 42 - DNA, 369 bp, artificial sequence
  D-Ye-29 VHH chain nucleotide sequence
caggtgcagctgcaggagtctgggggaggcttggtgcagcctggggggtctctgagactctcctgtgcagcctctggaagcgagttcagtttcattcccacgggctggtaccgccagactccagggaagcagcgcgacttggtcgcagtttttacgagtggcggtctcacaaactatgcagactccgtgaagggccgattcaccatctccagaaacaacaccaagaacatagtgtatctgcaaatgaacagcctcaaacctgaggacacggccgtctattactgtagtggagtcccaggtccacactacaatggtccgacatcggggataaactactggggccaggggacccaggtcaccgtctccagt

SEQ ID NO: 43 - DNA, 357 bp, artificial sequence
  D-Ye-31 VHH chain nucleotide sequence
caggtgcagctgcaggagtctggaggaggattggtgcaggctgggggctctctgggactctcctgcgcagcctctggacgcaccttcagtagcatgaccatcggctggttccgccaaactccagggaaggagcgtgagtttgtagcaggtattgggtggagtacgagtaaaacagtctacaaagactccgtgaagggccgattcaccatttccacagacaatgccaagaaaacggtgtatctgcaaatgaacaacctgaaacctgaggacacggccgtttattactgtgcagcagattcaatgaatagaggacagtttgactactggggccaggggacccaggtcaccgtctccagt

SEQ ID NO: 44 - DNA, 336 bp, artificial sequence
  D-Ye-32 VHH chain nucleotide sequence
caggtgcagctgcaggagtctggaggaggcttggtgcaggctggggggtctctgagactctcctgtgcagcctctgggagcgtcggcagtatcaatgccatggcctggttccgccaggcgccagggaagcagcgcgacgtggtcgcacatatgccttctggtggtagcacacactatgcagactccgtgaagggccgattcaccgtctccagagacaacgccaagaacacggtgtatctacaaatgaacagcctgaaagctgaggacacggccgtctattactgttgggcagctggtctggggtggggccaggggacccaggtcaccgtctccagt

SEQ ID NO: 45 - DNA, 369 bp, artificial sequence
  HZ-D-Ye-29-3 VHH chain nucleotide sequence
gaggtgcagctgctggagagcggaggcggactggtgcagcccggaggatctctgagactgagctgtgctgctagtgggagcgagttctcttttatccccacaggatggtacagacaggcccctggaaaacagagagagctggtggctgtgtttacctctggagggctgaccaactacgccgactctgtgaaagggaggtttactatcagcagggacaacagcaagaacacagtgtatctccagatgaacagtctgagagccgaagacaccgccgtctattattgcagcggcgtgccaggacctcattacaacgggcctaccagcggcatcaactactggggacagggcacccaggtgacagtgtcatcc

SEQ ID NO: 46 - DNA, 357 bp, artificial sequence
  HZ-D-Na-96-1 VHH chain nucleotide sequence
gaggtgcagctggtggagagcggaggaggactggtgcagcccggcggctctctgagactgagctgcgccgcctccggaaggacctttagctccatgaccatcggctggttcagacaagcccccggcaagggactggagttcgtgagcggcatcggctggacaagcggactgaccgtgtatgccgacagcgtcaagggaaggttcaccatctctagggacaacgccaagaacagcatgtatctgcagatgaactctctgagggccgaggacaccgccgtgtactactgcgccgccgacagcatgaacagaggccagttcgactactggggccaaggcacactggtgacagtgagcagc

SEQ ID NO: 47 - DNA, 357 bp, artificial sequence
  HZ-D-Na-96-2 VHH chain nucleotide sequence
gaggtgcagctggtggaaagcggcggaggactggtgcagcccggcggatctctgagactcagctgtgctgccagcggaaggaccttcagcagcatgaccatcggctggttcagacaagcccccggcaagggactggagttcgtgagcggcatcggctggacaagcggactgaccgtgtatgccgacagcgtcaagggaaggttcaccatctctagggacaatgccaagaactctctgtatctgcagatgaactctctgaagcccgaggataccgccgtgtactactgcgccgccgatagcatgaataggggccagttcgactactggggccaaggcacactggtgacagtgagcagc

SEQ ID NO: 48 - DNA, 357 bp, artificial sequence
  HZ-D-Na-96-3 VHH chain nucleotide sequence
gaggtgcagctggtggaaagcggcggaggactggtgcagcccggcggatctctgagactgagctgcgccgccagcggaaggaccttctccagcatgaccatcggctggtttaggcaagcccccggcaaggagagagagttcgtgagcggcatcggctggacaagcggactgaccgtgtacgccgatagcgtgaagggaaggttcaccatctctagggacaacgccaagaactccatgtatctgcagatgaactctctgaagcccgaggataccgccgtgtactactgcgccgccgacagcatgaacagaggccagttcgactactggggccaaggcacactggtgacagtgtccagc

SEQ ID NO: 49 - DNA, 372 bp, artificial sequence
  K-Yr-13&14-02 VHH chain nucleotide sequence
caagtgcagctggtagagtctgggggaggattggtcaaggctggggactctctgagactctcctgtgcagcctctggacacaccttcattatttatgccattggctggttccgccaggctccagggaaggagcgtgagtttgtagcaactattaactggagtggtagtatgacaaactatacagactccgtgaagggccgattcaccatctccagagacaacgccaagaacacggtgtatctccaaatgaacagcctgaaacctgacgacacggccatttattactgtgcggcttacgtcggtgcgactatttccaccgcccattcccgatatgactactggggccagggaacccaggtcaccgtgtcctca

SEQ ID NO: 50 - DNA, 372 bp, artificial sequence
  K-Yr-13&14-09 VHH chain nucleotide sequence
caagtgcagctggtggagtctgggggaggattggtcaaggctggggactctctgagactctcctgtgcagcctctggacgcaccttcactatttatgccattggctggttccgccaggctccagggaaggagcgtgagtttgtagcaactattaactggagtggtagtatgacaaactatacagactccgtgaagggccgattcaccatctccagagacaacgccaagaacacggtgtatctccaaatgaacagcctgaaacctgacgacacggccatttattactgtgcggcttacgtcggtgcgactatttccaccgcccattcccgatatgactactggggccaggggaccctggtcactgtctccgca

SEQ ID NO: 51 - DNA, 372 bp, artificial sequence
  K-Yr-13&14-16 VHH chain nucleotide sequence
gaagtgcagctggtggagtctgggggaggattggtgcaggctgggggctctctgagactctcctgtgcagcctctacacgcaccttcattacctatgccatgggctggttccgccaggctccagggaaggagcgtgagtttgtagcatctattaactggagtggtgctagcacatactatgcagactccgtgaagggccgattcaccatctccagacacaacgccaagaacacggtgtatctgcaaatgaacagcctgaaacctgaggacacggccgtttattactgtgcagcagctttgtcagcagtagtagttacacagatcctagactatgactactggggccaggggaccctggtcaccgtctcctca

SEQ ID NO: 52 - DNA, 372 bp, artificial sequence
  HZ-K-Yr-13&14-02-3 VHH chain nucleotide sequence
caagtgcagctggtggagagcggaggaggactggtgaagcccggcggctctctgagactgagctgtgccgcctccggccacaccttcatcatctacgccatcggctggtttaggcaagcccccggcaaaggactggagttcgtggccaccatcaactggagcggcagcatgaccaactacgccgactccgtgaagggaaggttcacaatctctagggacaacgccaagaacaccgtgtatctgcagatgaactctctgaagcccgacgacaccgccgtgtactactgcgctgcctatgtgggcgccaccatcagcacagcccacagcagatacgactactggggacaaggcacactggtgaccgtgagcagc

SEQ ID NO: 53 - DNA, 1470 bp, artificial sequence
  Bi-201 nucleotide sequence
caagtgcagctggtggagagcggaggaggactggtgaagcccggcggctctctgagactgagctgtgccgcctccggccacaccttcatcatctacgccatcggctggtttaggcaagcccccggcaaaggactggagttcgtggccaccatcaactggagcggcagcatgaccaactacgccgactccgtgaagggaaggttcacaatctctagggacaacgccaagaacaccgtgtatctgcagatgaactctctgaagcccgacgacaccgccgtgtactactgcgctgcctatgtgggcgccaccatcagcacagcccacagcagatacgactactggggacaaggcacactggtgaccgtgagcagcgacaaaacccatacatgtcctccttgccccgcccctgaggctgctggaggccccagcgtgttcctgtttccccccaagcccaaagataccctcatgatctccaggacccccgaagtgacctgcgtcgtggtcgacgtgagccacgaggaccctgaagtcaagttcaactggtacgtcgatggcgtggaggtgcacaacgctaagaccaaaccccgggaagagcagtacaattccacctacagggtggtgtccgtcctgacagtgctgcaccaagactggctgaatggaaaggagtacaagtgcaaagtgagcaataaggccctccctgctcccattgagaagaccatttccaaggccaaaggccagcctcgggaaccccaggtgtacacactgcccccttccagggaggagatgaccaagaaccaggtgagcctcacctgcctggtgaagggcttctaccctagcgacattgctgtggagtgggagagcaacggccagcccgaaaacaactataagacaacccctcccgtgctggacagcgacggctccttctttctgtactccaagctcaccgtggacaagtccaggtggcaacagggaaacgtgttctcctgctccgtgatgcacgaggccctccacaaccactacacccagaagagcctgagcctgtcccctggcggtggcggcggtagtggcggaggcgggagtggcggtggagggtcaggtggtggaggctcgggtgaggtgcagctggtggagagcggaggaggactggtgcagcccggcggctctctgagactgagctgcgccgcctccggaaggacctttagctccatgaccatcggctggttcagacaagcccccggcaagggactggagttcgtgagcggcatcggctggacaagcggactgaccgtgtatgccgacagcgtcaagggaaggttcaccatctctagggacaacgccaagaacagcatgtatctgcagatgaactctctgagggccgaggacaccgccgtgtactactgcgccgccgacagcatgaacagaggccagttcgactactggggccaaggcacactggtgacagtgagcagc

SEQ ID NO: 54 - DNA, 1470 bp, artificial sequence
  Bi-202 nucleotide sequence
caagtgcagctggtggagagcggaggaggactggtgaagcccggcggctctctgagactgagctgtgccgcctccggccacaccttcatcatctacgccatcggctggtttaggcaagcccccggcaaaggactggagttcgtggccaccatcaactggagcggcagcatgaccaactacgccgactccgtgaagggaaggttcacaatctctagggacaacgccaagaacaccgtgtatctgcagatgaactctctgaagcccgacgacaccgccgtgtactactgcgctgcctatgtgggcgccaccatcagcacagcccacagcagatacgactactggggacaaggcacactggtgaccgtgagcagcggcggtggcggcggtagtggcggaggcgggagtggcggtggagggtcaggtggtggaggctcgggtgaggtgcagctggtggagagcggaggaggactggtgcagcccggcggctctctgagactgagctgcgccgcctccggaaggacctttagctccatgaccatcggctggttcagacaagcccccggcaagggactggagttcgtgagcggcatcggctggacaagcggactgaccgtgtatgccgacagcgtcaagggaaggttcaccatctctagggacaacgccaagaacagcatgtatctgcagatgaactctctgagggccgaggacaccgccgtgtactactgcgccgccgacagcatgaacagaggccagttcgactactggggccaaggcacactggtgacagtgagcagcgacaaaacccatacatgtcctccttgccccgcccctgaggctgctggaggccccagcgtgttcctgtttccccccaagcccaaagataccctcatgatctccaggacccccgaagtgacctgcgtcgtggtcgacgtgagccacgaggaccctgaagtcaagttcaactggtacgtcgatggcgtggaggtgcacaacgctaagaccaaaccccgggaagagcagtacaattccacctacagggtggtgtccgtcctgacagtgctgcaccaagactggctgaatggaaaggagtacaagtgcaaagtgagcaataaggccctccctgctcccattgagaagaccatttccaaggccaaaggccagcctcgggaaccccaggtgtacacactgcccccttccagggaggagatgaccaagaaccaggtgagcctcacctgcctggtgaagggcttctaccctagcgacattgctgtggagtgggagagcaacggccagcccgaaaacaactataagacaacccctcccgtgctggacagcgacggctccttctttctgtactccaagctcaccgtggacaagtccaggtggcaacagggaaacgtgttctcctgctccgtgatgcacgaggccctccacaaccactacacccagaagagcctgagcctgtcccct

SEQ ID NO: 55 - DNA, 1356 bp, artificial sequence
  Bi-203 nucleotide sequence
caagtgcagctggtggagagcggaggaggactggtgaagcccggcggctctctgagactgagctgtgccgcctccggccacaccttcatcatctacgccatcggctggtttaggcaagcccccggcaaaggactggagttcgtggccaccatcaactggagcggcagcatgaccaactacgccgactccgtgaagggaaggttcacaatctctagggacaacgccaagaacaccgtgtatctgcagatgaactctctgaagcccgacgacaccgccgtgtactactgcgctgcctatgtgggcgccaccatcagcacagcccacagcagatacgactactggggacaaggcacactggtgaccgtgagcagcgccagcacaaagggcccttccgtcttccctctggccccctccagcaagtccacaagcggaggaaccgctgccctcggctgcctcgtgaaagactatttccctgagcccgtgacagtgagctggaatagcggcgctctcacctccggagtccacaccttccccgctgtgctgcagagcagcggactgtatagcctgagctccgtggtgaccgtgcctagctcctccctcggcacccagacctacatttgcaatgtgaaccacaagcctagcaacaccaaggtggacaagaaggtggagcccaagagctgcgacaaaacccatacatgtcctccttgccccgcccctgaggctgctggaggccccagcgtgttcctgtttccccccaagcccaaagataccctcatgatctccaggacccccgaagtgacctgcgtcgtggtcgacgtgagccacgaggaccctgaagtcaagttcaactggtacgtcgatggcgtggaggtgcacaacgctaagaccaaaccccgggaagagcagtacaattccacctacagggtggtgtccgtcctgacagtgctgcaccaagactggctgaatggaaaggagtacaagtgcaaagtgagcaataaggccctccctgctcccattgagaagaccatttccaaggccaaaggccagcctcgggaaccccaggtgtacacactgcccccttccagggaggagatgaccaagaaccaggtgagcctcacctgcctggtgaagggcttctaccctagcgacattgctgtggagtgggagagcaacggccagcccgaaaacaactataagacaacccctcccgtgctggacagcgacggctccttctttctgtactccaagctcaccgtggacaagtccaggtggcaacagggaaacgtgttctcctgctccgtgatgcacgaggccctccacaaccactacacccagaagagcctgagcctgtcccct

SEQ ID NO: 56 - DNA, 678 bp, artificial sequence
  Bi-204 nucleotide sequence
gaggtgcagctggtggagagcggaggaggactggtgcagcccggcggctctctgagactgagctgcgccgcctccggaaggacctttagctccatgaccatcggctggttcagacaagcccccggcaagggactggagttcgtgagcggcatcggctggacaagcggactgaccgtgtatgccgacagcgtcaagggaaggttcaccatctctagggacaacgccaagaacagcatgtatctgcagatgaactctctgagggccgaggacaccgccgtgtactactgcgccgccgacagcatgaacagaggccagttcgactactggggccaaggcacactggtgacagtgagcagccggaccgtggccgccccttccgtgttcatctttcccccctccgacgagcagctgaagtccggaaccgccagcgtggtgtgcctcctgaacaacttttacccccgggaggccaaggtgcagtggaaggtggacaacgccctgcaaagcggcaactcccaggaatccgtcaccgagcaggattccaaggattccacctacagcctgtcctccaccctgacactgtccaaggccgactacgagaagcacaaggtgtacgcctgcgaggtgacacaccagggcctgagcagccccgtgaccaagtccttcaaccggggcgagtgt

SEQ ID NO: 57 - protein, 8 aa, artificial sequence
  D-Na-96 CDR1
GRTFSSMT

SEQ ID NO: 58 - protein, 9 aa, artificial sequence
  D-Na-96 CDR2
GIGWTSGLT

SEQ ID NO: 59 - protein, 12 aa, artificial sequence
  D-Na-96 CDR3
AADSMNRGQFDY

SEQ ID NO: 60 - protein, 8 aa, artificial sequence
  D-Ye-29 CDR1
GSEFSFIP

SEQ ID NO: 61 - protein, 8 aa, artificial sequence
  D-Ye-29 CDR2
VFTSGGLT

SEQ ID NO: 62 - protein, 17 aa, artificial sequence
  D-Ye-29 CDR3
SGVPGPHYNGPTSGINY

SEQ ID NO: 63 - protein, 8 aa, artificial sequence
  K-Yr-13&14-02 CDR1
GHTFIIYA

SEQ ID NO: 64 - protein, 8 aa, artificial sequence
  K-Yr-13&14-02 CDR2
INWSGSMT

SEQ ID NO: 65 - protein, 17 aa, artificial sequence
  K-Yr-13&14-02 CDR3
AAYVGATISTAHSRYDY

SEQ ID NO: 66 - DNA, 23 bp, artificial sequence
  primer
gtcctggctgctcttctacaagg

SEQ ID NO: 67 - DNA, 23 bp, artificial sequence
  primer
ggtacgtgctgttgaactgttcc

SEQ ID NO: 68 - DNA, 33 bp, artificial sequence
  primer
ctagtgcggccgcctggagacggtgacctgggt

SEQ ID NO: 69 - DNA, 38 bp, artificial sequence
  primer
cgcggatcccaggtgcagctgcaggagtctggrggagg

SEQ ID NO: 70 - DNA, 89 bp, artificial sequence
  primer
atttttactgctgttttattcgcagcatcctccgcattagctaaaagagaggctgaagcacaggtgcagctgcaggagtctggrggagg

SEQ ID NO: 71 - DNA, 81 bp, artificial sequence
  primer
agttgtcagttcctgtgccccccctcctcccgcgccacctccgcccgcacctccgccaccactggagacggtgacctgggt